European Patent Specification EP 3 839 514 B1, published December 13, 2023. Title: IMMUNOASSAY FOR THE DETECTION OF CLEAVED HIGH MOLECULAR WEIGHT KININOGEN. Applicant: Dyax Corp. Application Not Yet Assigned. The sequence listing filed with the application follows.

SEQUENCE LISTING (83 sequences)

SEQ ID NO: 1 - protein, 644 aa, Homo sapiens
MKLITILFLCSRLLLSLTQESQSEEIDCNDKDLFKAVDAALKKYNSQNQSNNQFVLYRITEATKTVGSDTFYSFKYEIKEGDCPVQSGKTWQDCEYKDAAKAATGECTATVGKRSSTKFSVATQTCQITPAEGPVVTAQYDCLGCVHPISTQSPDLEPILRHGIQYFNNNTQHSSLFMLNEVKRAQRQVVAGLNFRITYSIVQTNCSKENFLFLTPDCKSLWNGDTGECTDNAYIDIQLRIASFSQNCDIYPGKDFVQPPTKICVGCPRDIPTNSPELEETLTHTITKLNAENNATFYFKIDNVKKARVQVVAGKKYFIDFVARETTCSKESNEELTESCETKKLGQSLDCNAEVYVVPWEKKIYPTVNCQPLGMISLMKRPPGFSPFRSSRIGEIKEETTVSPPHTSMAPAQDEERDSGKEQGHTRRHDWGHEKQRKHNLGHGHKHERDQGHGHQRGHGLGHGHEQQHGLGHGHKFKLDDDLEHQGGHVLDHGHKHKHGHGHGKHKNKGKKNGKHNGWKTEHLASSSEDSTTPSAQTQEKTEGPTPIPSLAKPGVTVTFSDFQDSDLIATMMPPISPAPIQSDDDWIPDIQIDPNGLSFNPISDFPDTTSPKCPGRPWKSVSEINPTTQMKESYYFDLTDGLS

SEQ ID NO: 2 - protein, 362 aa, Homo sapiens
QESQSEEIDCNDKDLFKAVDAALKKYNSQNQSNNQFVLYRITEATKTVGSDTFYSFKYEIKEGDCPVQSGKTWQDCEYKDAAKAATGECTATVGKRSSTKFSVATQTCQITPAEGPVVTAQYDCLGCVHPISTQSPDLEPILRHGIQYFNNNTQHSSLFMLNEVKRAQRQVVAGLNFRITYSIVQTNCSKENFLFLTPDCKSLWNGDTGECTDNAYIDIQLRIASFSQNCDIYPGKDFVQPPTKICVGCPRDIPTNSPELEETLTHTITKLNAENNATFYFKIDNVKKARVQVVAGKKYFIDFVARETTCSKESNEELTESCETKKLGQSLDCNAEVYVVPWEKKIYPTVNCQPLGMISLMK

SEQ ID NO: 3 - protein, 255 aa, Homo sapiens
SSRIGEIKEETTVSPPHTSMAPAQDEERDSGKEQGHTRRHDWGHEKQRKHNLGHGHKHERDQGHGHQRGHGLGHGHEQQHGLGHGHKFKLDDDLEHQGGHVLDHGHKHKHGHGHGKHKNKGKKNGKHNGWKTEHLASSSEDSTTPSAQTQEKTEGPTPIPSLAKPGVTVTFSDFQDSDLIATMMPPISPAPIQSDDDWIPDIQIDPNGLSFNPISDFPDTTSPKCPGRPWKSVSEINPTTQMKESYYFDLTDGLS

SEQ ID NO: 4 - protein, 123 aa, Artificial Sequence
  Synthetic Polypeptide
EVQLLESGGGLVQPGGSLRLSCAASGFTFSFYVMVWVRQAPGKGLEWVSGISPSGGNTAYADSVKGRFTISRDNSKNTLYLQMNSLRAEDTAVYYCARKLFYYDDTKGYFDFWGQGTLVTVSS

SEQ ID NO: 5 - protein, 110 aa, Artificial Sequence
  Synthetic Polypeptide
QYELTQPPSASGTPGQRVTLSCSGSSSNIGSNYVYWYQQLPGTAPKLLIYRNNQRPSGVPDRFSGSKSGTSASLAISGLQSEDEADYYCAAWDDSLNGRVFGGGTKLTVL

SEQ ID NO: 6 - protein, 120 aa, Artificial Sequence
  Synthetic Polypeptide
EVQLLESGGGLVQPGGSLRLSCAASGFTFSLYPMVWVRQAPGKGLEWVSSIYPSGGFTTYADSVKGRFTISRDNSKNTLYLQMNSLRAEDTAVYYCARSSRYYYYGMDVWGQGTTVTVSS

SEQ ID NO: 7 - protein, 110 aa, Artificial Sequence
  Synthetic Polypeptide
QYELTQPPSMSGTPGQRVTISCSGSSSNIGSEYVYWFQQLPGTAPKLLIYRNDQRPSGVPDRFSGSKSGTSASLAISGLRSEDETDYYCSTWDDTLRTGVFGGGTKVTVL

SEQ ID NO: 8 - protein, 118 aa, Artificial Sequence
  Synthetic Polypeptide
EVQLLESGGGLVQPGGSLRLSCAASGFTFSRYRMRWVRQAPGKGLEWVSGISPSGGWTYYADSVKGRFTISRDNSKNTLYLQMNSLRAEDTAVYYCTTDNGDYALAHWGQGTLVTVSS

SEQ ID NO: 9 - protein, 108 aa, Artificial Sequence
  Synthetic Polypeptide
QDIQMTQSPSSLSASVGDRVTITCRASQRIINYLNWYQQKPGKAPKLLIYAASSLQSGVPSRFSGSGSGTDFTLTISSLQPEDFATYYCQQSYSAPLTFGGGTRVEIK

SEQ ID NO: 10 - protein, 125 aa, Artificial Sequence
  Synthetic Polypeptide
EVQLLESGGGLVQPGGSLRLSCAASGFTFSQYSMGWVRQAPGKGLEWVSSIYSSGGSTQYADSVKGRFTISRDNSKNTLYLQMNSLRAEDTATYYCARTRRGWFGEDYYYYMDVWGKGTTVTVSS

SEQ ID NO: 11 - protein, 108 aa, Artificial Sequence
  Synthetic Polypeptide
QDIQMTQSPSSLSASVGDRITITCRASQGIRNDVGWYQQKPGKAPQRLIYAASSLQSGVPSRFSGSGSGTEFTLTISSLQPEDFATYYCLQHNSYPLTFGGGTKVEIK

SEQ ID NO: 12 - protein, 126 aa, Artificial Sequence
  Synthetic Polypeptide
EVQLLESGGGLVQPGGSLRLSCAASGFTFSPYMMYWVRQAPGKGLEWVSSISPSGGKTWYADSVKGRFTISRDNSKNTLYLQMNSLRAEDTAVYYCARLGGSSSYYYYYYYGMDVWGQGTTVTVSS

SEQ ID NO: 13 - protein, 111 aa, Artificial Sequence
  Synthetic Polypeptide
QSALTQSPSASGTPGQRVTISCSGSSSNIGGNTVNWYQQFPGTAPKLLIYSNNQRPSGVPDRFSGSKSGTSASLAISGLQSEDEAIYYCASWDDRLNGHWVFGGGTRLTVL

SEQ ID NO: 14 - protein, 123 aa, Artificial Sequence
  Synthetic Polypeptide
EVQLLESGGGLVQPGGSLRLSCAASGFTFSAYDMHWVRQAPGKGLEWVSSIWPSGGGTYYADSVKGRFTISRDNSKNTLYLQMNSLRAEDTAVYYCARGDYDYGDFTDAFDIWGQGTMVTVSS

SEQ ID NO: 15 - protein, 110 aa, Artificial Sequence
  Synthetic Polypeptide
QSALTQPASVSGSPGQSITISCTGTSSDVGSYNLVSWYQQHPGKAPKLMIYEGSKRPSGVPDRFSGSKSGNTASLIISGLQAEDEADYYCCSYAGSYSYVFGTGTRVTVL

SEQ ID NO: 16 - protein, 118 aa, Artificial Sequence
  Synthetic Polypeptide
EVQLLESGGGLVQPGGSLRLSCAASGFTFSNYAMQWVRQAPGKGLEWVSWIYSSGGPTYYADSVKGRFTISRDNSKNTLYLQMNSLRAEDTAVYYCARGLPGQPFDYWGQGTLVTVSS

SEQ ID NO: 17 - protein, 110 aa, Artificial Sequence
  Synthetic Polypeptide
QSELTQPPSASGTPGQRVTISCSGSSSNIGNNYVYWYQQFPGTAPKLLIYRNNQRPSGVPDRFSGSKSGTSASLAISGLRSEDEADYYCATWDDRLSGWVFGGGTKLTVL

SEQ ID NO: 18 - protein, 116 aa, Artificial Sequence
  Synthetic Polypeptide
EVQLLESGGGLVQPGGSLRLSCAASGFTFSSYQMHWVRQAPGKGLEWVSGIYSSGGSTPYADSVKGRFTISRDNSKNTLYLQMNSLRAEDTAVYYCARGHHGMDVWGQGTTVTVSS

SEQ ID NO: 19 - protein, 108 aa, Artificial Sequence
  Synthetic Polypeptide
QDIQMTQSPSSVSASVGDRVTITCRASQGISSWLAWYQQKPGKAPKLLIYAASNLQSGVPSRFSGSGSGTDFTLTISSLQPEDFATYYCQKYNIAPYTFGQGTKLEIK

SEQ ID NO: 20 - protein, 120 aa, Artificial Sequence
  Synthetic Polypeptide
EVQLLESGGGLVQPGGSLRLSCAASGFTFSPYPMTWVRQAPGKGLEWVSGISSSGGFTPYADSVKGRFTISRDNSKNTLYLQMNSLRAEDTAVYYCARMVRGVIKAFDIWGQGTMVTVSS

SEQ ID NO: 21 - protein, 110 aa, Artificial Sequence
  Synthetic Polypeptide
QYELTQPPSASGTPGQRVTISCSGSSSNIGSHYVFWYQQLPGAAPKLLIYRNNQRPSGVPDRFSGSKSGTSASLAISGLRSEDEADYYCATWDNSLSAWVFGGGTKLTVL

SEQ ID NO: 22 - protein, 117 aa, Artificial Sequence
  Synthetic Polypeptide
EVQLLESGGGLVQPGGSLRLSCAASGFTFSKYTMWWVRQAPGKGLEWVSVISSSGGKTYYADSVKGRFTISRDNSKNTLYLQMNSLRAEDTAVYYCARTANRAFDIWGQGTMVTVSS

SEQ ID NO: 23 - protein, 108 aa, Artificial Sequence
  Synthetic Polypeptide
QDIQMTQSPAALSVSPGERATLSCRASQSVSSDLAWYQQKPGQAPRLLIHGASTRATGIPARFSGSGSGREFTLTISSLQSEDFAVYYCQQYNDWPPLFGPGTKVNIK

SEQ ID NO: 24 - protein, 125 aa, Artificial Sequence
  Synthetic Polypeptide
EVQLLESGGGLVQPGGSLRLSCAASGFTFSRYYMAWVRQAPGKGLEWVSGIVPSGGQTGYADSVKGRFTISRDNSKNTLYLQMNSLRAEDTAVYYCARTRRGWFGEDYYYYMDVWGKGTLVTVSS

SEQ ID NO: 25 - protein, 111 aa, Artificial Sequence
  Synthetic Polypeptide
QDIQMTQSPGTLSLSPGERATVSCRASQSVGSTYLAWYQHKPGQAPRLLIYGASSRATGIPDRFSGSGSGTDFTLTISSLEPEDFAIYYCQHFHTSPPGITFGQGTRLEIK

SEQ ID NO: 26 - protein, 118 aa, Artificial Sequence
  Synthetic Polypeptide
EVQLLESGGGLVQPGGSLRLSCAASGFTFSMYKMSWVRQAPGKGLEWVSVISPSGGRTYYADSVKGRFTISRDNSKNTLYLQMNSLRAEDTAVYYCARGTRTSGLDYWGQGTLVTVSS

SEQ ID NO: 27 - protein, 110 aa, Artificial Sequence
  Synthetic Polypeptide
QSALTQPASVSGSPGQSITISCTGTSSDVGGYKYVSWYQQHPGKAPKLVIYEVSNRPSGVSNRFSGSKSGNTASLTISGLQAEDEADYYCSSYTSSTTVVFGGGTKLTVL

SEQ ID NO: 28 - protein, 119 aa, Artificial Sequence
  Synthetic Polypeptide
EVQLLESGGGLVQPGGSLRLSCAASGFTFSTYGMRWVRQAPGKGLEWVSVISPSGGKTNYADSVKGRFTISRDNSKNTLYLQMNSLRAEDTAVYYCARGRPDYYAMDVWGQGTTVTVSS

SEQ ID NO: 29 - protein, 110 aa, Artificial Sequence
  Synthetic Polypeptide
QSALTQPPSASGAPGQRVTISCSGSSSNIGSNTVNWYQKLPGTAPKLLIYYNDRRPSGVPDRFSGSKSGNTASLTISGLQAEDEADYYCAAWDDSLSGPVFGGGTKLTVL

SEQ ID NO: 30 - protein, 126 aa, Artificial Sequence
  Synthetic Polypeptide
EVQLLESGGGLVQPGGSLRLSCAASGFTFSIYPMSWVRQAPGKGLEWVSGISPSGGKTAYADSVKGRFTISRDNSKNTLYLQMNSLRAEDTAVYYCARGQGRAVRGKLYYYGMDVWGQGTTVTVSS

SEQ ID NO: 31 - protein, 110 aa, Artificial Sequence
  Synthetic Polypeptide
QSALTQPPSASQTPGQTVTISCSGSSSNIGTNNVNWYQQLPGTAPKLLISSHHRRPSGVPDRFSASKSGTSASLAISGLQSEDEADYYCAAWDDSLNGPVFGGGTKLTVL

SEQ ID NO: 32 - protein, 117 aa, Artificial Sequence
  Synthetic Polypeptide
EVQLLESGGGLVQPGGSLRLSCAASGFTFSMYHMNWVRQAPGKGLEWVSSIYSSGGSTRYADSVKGRFTISRDNSKNTLYLQMNSLRAEDTAVYYCARGVRYGMDVWGQGTTVTVSS

SEQ ID NO: 33 - protein, 108 aa, Artificial Sequence
  Synthetic Polypeptide
QDIQMTQSPSSVSASVGDRVTITCRASQGISSWLAWYQQKPGKAPKLLIYAASSLQSGVPSRFSGSGSGTDFTLTISSLQPEDFATYYCQQANSFPITFGQGTRLEIK

SEQ ID NO: 34 - protein, 122 aa, Artificial Sequence
  Synthetic Polypeptide
EVQLLESGGGLVQPGGSLRLSCAASGFTFSMYDMHWVRQAPGKGLEWVSSISSSGGYTQYADSVKGRFTISRDNSKNTLYLQMNSLRAEDTAMYYCARDRGLIAAAGGFDPWGQGTLVTVSS

SEQ ID NO: 35 - protein, 108 aa, Artificial Sequence
  Synthetic Polypeptide
QDIQMTQSPSSLSASVGDRVTITCRASQSIGIYLNWYQQKPGTAPKLLIYAASSLQSGVPSRFTGSGSGTDFTLTISSLQPDDFATYYCQRTYGRPLTFGGGTKVEIK

SEQ ID NO: 36 - protein, 121 aa, Artificial Sequence
  Synthetic Polypeptide
EVQLLESGGGLVQPGGSLRLSCAASGFTFSKYEMMWVRQAPGKGLEWVSSISPSGGYTMYADSVKGRFTISRDNSKNTLYLQMNSLRAEDTAVYYCARHRSKWNDAPFDSWGQGTLVTVSS

SEQ ID NO: 37 - protein, 109 aa, Artificial Sequence
  Synthetic Polypeptide
QDIQMTQSPSSLSASVGDRVAITCRASQSIDTYLNWYQQKPGKAPKLLIYAASKLEDGVPSRFSGSGTGTDFTLTIRSLQPEDFASYFCQQSYSSPGITFGPGTKVEIK

SEQ ID NO: 38 - protein, 123 aa, Artificial Sequence
  Synthetic Polypeptide
EVQLLESGGGLVQPGGSLRLSCAASGFTFSIYQMYWVRQAPGKGLEWVSSIYSSGGRTFYADSVKGRFTISRDNSKNTLYLQMNSLRAEDTAVYYCATRGSWYVGGNEYFQHWGQGTLVTVSS

SEQ ID NO: 39 - protein, 106 aa, Artificial Sequence
  Synthetic Polypeptide
QSVLTQSPSLSLSPGQTASIPCSGDTLGNKFVSWYQQKPGQSPVLVIYQDTKRPSGIPERFSGSNSGNTATLTITGTQAMDEADYYCQVWDSNSYAFGPGTKVTVL

SEQ ID NO: 40 - protein, 120 aa, Artificial Sequence
  Synthetic Polypeptide
EVQLLESGGGLVQPGGSLRLSCAASGFTFSFYMMYWVRQAPGKGLEWVSSISSSGGFTRYADSVKGRFTISRDNSKNTLYLQMNSLRAEDTAVYYCARVRGLAVAAPDYWGQGTLVTVSS

SEQ ID NO: 41 - protein, 110 aa, Artificial Sequence
  Synthetic Polypeptide
QSELTQPASVSGSPGQSITISCIGTSSDIGTYNYVSWYQQHPGKAPKLMIYDVNTRPSGVSDRFSGSKSGNTASLTISGLQAEDEADYYCSSYTTSVTWVFGGGTTLTVL

SEQ ID NO: 42 - protein, 115 aa, Artificial Sequence
  Synthetic Polypeptide
EVQLLESGGGLVQPGGSLRLSCAASGFTFSGYNMYWVRQAPGKGLEWVSRISPSGGWTSYADSVKGRFTISRDNSKNTLYLQMNSLRAEDTAVYYCTRGQWMDWWGQGTMVTVSS

SEQ ID NO: 43 - protein, 108 aa, Artificial Sequence
  Synthetic Polypeptide
QDIQMTQSPSSLSASVGDRVIITCRASQNITGYLNWYQQKPGKAPNLLIYDASRMNTGVPSRFRGSGSGTDYILTIYKLEPEDIGTYFCQHTDDFSVTFGGGTKVDLK

SEQ ID NO: 44 - protein, 116 aa, Artificial Sequence
  Synthetic Polypeptide
EVQLLESGGGLVQPGGSLRLSCAASGFTFHYRMMWVRQAPGKGLEWVSYISSSGGYTAYADSVKGRFTISRDNSKNTLYLQMNSLRAEDTAVYYCAAKRNRAFDIWGQGTMVTVSS

SEQ ID NO: 45 - protein, 114 aa, Artificial Sequence
  Synthetic Polypeptide
QDIQMTQSPDSLAVSLGERATINCKSSQSVLYSSNNKNYLAWYQQKPGQPPKLLIYWASTRESGVPDRFSGSGSGTDFTLTISSLQAEDVAVYYCQQYYSTPLGFGQGTKLEIK

SEQ ID NO: 46 - protein, 120 aa, Artificial Sequence
  Synthetic Polypeptide
EVQLLESGGGLVQPGGSLRLSCAASGFTFSRYQMTWVRQAPGKGLEWVSSIGSSGGFTNYADSVKGRFTISRDNSKNTLYLQMNSLRAEDTAVYYCARLPANFYYYMDVWGKGTTVTVSS

SEQ ID NO: 47 - protein, 108 aa, Artificial Sequence
  Synthetic Polypeptide
QDIQMTQSPSSLSASVGDRVTITCRASQNIYSFLNWYQQKPGKAPKLLIYATSSLQSGVPSRFSGSGSGTDFTLTISSLQPEDFASYYCQQNYNIPWTFGQGTKVEIK

SEQ ID NO: 48 - protein, 123 aa, Artificial Sequence
  Synthetic Polypeptide
EVQLLESGGGLVQPGGSLRLSCAASGFTFSWYMMKWVRQAPGKGLEWVSSIVPSGGWTTYADSVKGRFTISRDNSKNTLYLQMNSLRAEDTAVYYCATEGNLWFGEGRAFDIWGQGTMVTVSS

SEQ ID NO: 49 - protein, 109 aa, Artificial Sequence
  Synthetic Polypeptide
QDIQMTQSPGTLSLSPGERATLSCRASQSVSSSYLAWYQQKPGQAPRLLIYGASSRATGIPDRFSGSGSGTDFTLTISRLEPEDFAVYYCQQRSNWPPSFGQGTRLDIK

SEQ ID NO: 50 - protein, 126 aa, Artificial Sequence
  Synthetic Polypeptide
EVQLLESGGGLVQPGGSLRLSCAASGFTFSKYDMHWVRQAPGKGLEWVSRISSSGGKTEYADSVKGRFTISRDNSKNTLYLQMNSLRAEDTAVYYCAREYRYCTANTCSLYGMDVWGRGTTVTVSS

SEQ ID NO: 51 - protein, 108 aa, Artificial Sequence
  Synthetic Polypeptide
QDIQMTQSPSSLSASVGDRVAITCRTSQGVRSDFAWYQQTPGKAPRRLIYAAFILDNGVPSRFSGSGSGTEFTLTISSLQPEDFATYYCQQSYSTPLTFGGGTKVEMK

SEQ ID NO: 52 - protein, 120 aa, Artificial Sequence
  Synthetic Polypeptide
EVQLLESGGGLVQPGGSLRLSCAASGFTFSPYWMHWVRQAPGKGLEWVSVISPSGGGTGYADSVKGRFTISRDNSKNTLYLQMNSLRAEDTAVYYCARESRGSGSHEDYWGQGTLVTVSS

SEQ ID NO: 53 - protein, 109 aa, Artificial Sequence
  Synthetic Polypeptide
QDIQMTQSPATLSLSPGERATLSCRASQSVSSYLAWYQQKPGQAPRLLIYGASNRGTGIPARFSGSGSGTEFTLTISSLQSEDFAVYFCQQYKNWPNLTFGGGTKVDIK

SEQ ID NO: 54 - protein, 122 aa, Artificial Sequence
  Synthetic Polypeptide
EVQLLESGGGLVQPGGSLRLSCAASGFTFSHYPMAWVRQAPGKGLEWVSGIVSSGGRTVYADSVKGRFTISRDNSKNTLYLQMNSLRAEDTAVYYCARDPYDFWSEGAFDIWGQGTMVTVSS

SEQ ID NO: 55 - protein, 111 aa, Artificial Sequence
  Synthetic Polypeptide
QSVLTQPPSASGTPGQRVTISCSGSSSNIGNNFVYWYHQVPGTAPKLLIYKNNQRPSGVPDRFSGSKSAASASLAISGLRSEDEADYYCAAWDNSLSGFYVFGAGTKVTVL

SEQ ID NO: 56 - protein, 120 aa, Artificial Sequence
  Synthetic Polypeptide
EVQLLESGGGLVQPGGSLRLSCAASGFTFSWYGMHWVRQAPGKGLEWVSRIGPSGGPTSYADSVKGRFTISRDNSKNTLYLQMNSLRAEDTAVYYCARGYYGTGRYFQHWGQGTLVTVSS

SEQ ID NO: 57 - protein, 109 aa, Artificial Sequence
  Synthetic Polypeptide
QDIQMTQSPDSLSLSPGDRATLSCRASQSVGSDYLAWYQQKPGQAPRLLIYDASNRATGIPARFSGSGSGTDFTLTISSLEPEDFAVYYCQQRSNWPPTFGGGTKVEIK

SEQ ID NO: 58 - protein, 116 aa, Artificial Sequence
  Synthetic Polypeptide
EVQLLESGGGLVQPGGSLRLSCAASGFTFSAYAMRWVRQAPGKGLEWVSYISSSGGETMYADSVKGRFTISRDNSKNTLYLQMNSLRAEDTAVYYCANGYGRIDYWGQGTLVTVSS

SEQ ID NO: 59 - protein, 110 aa, Artificial Sequence
  Synthetic Polypeptide
QSVLTQPASVSGSPGQSITISCTGTSSDIGGYNYVSWYQQHPGKAPKLMIYEVSNRPSGVSNRFSGSKSGNTASLTISGLQAEDEADYYCSSYTSGSTRVFGTGTRVTVL

SEQ ID NO: 60 - protein, 121 aa, Artificial Sequence
  Synthetic Polypeptide
EVQLLESGGGLVQPGGSLRLSCAASGFTFSAYVMRWVRQAPGKGLEWVSSIGSSGGPTYYADSVKGRFTISRDNSKNTLYLQMNSLRAEDTAVYYCARRGGSGSSHAFDIWGQGTMVTVSS

SEQ ID NO: 61 - protein, 108 aa, Artificial Sequence
  Synthetic Polypeptide
QDIQMTQSPSSLSASVGDRVTITCRASQSISSYLNWYQQKPGKAPKLLIYAASSLQSGVPSRFSGSGSGTDFTLTISSLQPEDSGTYYCQQYNSFPLTFGGGTKVEIK

SEQ ID NO: 62 - protein, 122 aa, Artificial Sequence
  Synthetic Polypeptide
EVQLLESGGGLVQPGGSLRLSCAASGFTFSYYGMNWVRQAPGKGLEWVSVISPSGGLTVYADSVKGRFTISRDNSKNTLYLQMNSLRAEDTAMYYCATGFAVQHGGGAFDIWGQGTMVTVSS

SEQ ID NO: 63 - protein, 108 aa, Artificial Sequence
  Synthetic Polypeptide
QDIQMTQSPATLSMSPGERATLSCRASQSVTTYLAWYQQKPGQAPRLLIYDASIRATGVPARFSGSGSGTDFTLTISRLEPEDFAVYYCQQRTIWPLTFGGGTKVEIK

SEQ ID NO: 64 - protein, 119 aa, Artificial Sequence
  Synthetic Polypeptide
EVQLLESGGGLVQPGGSLRLSCAASGFTFSPYEMVWVRQAPGKGLEWVSSIVPSGGWTVYADSVKGRFTISRDNSKNTLYLQMNSLRAEDTAVYYCASPSGRGLAFDIWGQGTMVTVSS

SEQ ID NO: 65 - protein, 109 aa, Artificial Sequence
  Synthetic Polypeptide
QDIQMTQSPGTLSLSPGERATLSCRASQSISSSYLAWYQQKPGQAPRLLIYGASSRATGVPDRFSGSGSGTEFTLTISSLQPEDFATYYCLQQKSYPYTFGQGTKVEIK

SEQ ID NO: 66 - protein, 119 aa, Artificial Sequence
  Synthetic Polypeptide
EVQLLESGGGLVQPGGSLRLSCAASGFTFSKYFMTWVRQAPGKGLEWVSWISSSGGYTNYADSVKGRFTISRDNSKNTLYLQMNSLRAEDTAVYYCARGAYYYDAFDIWGQGTMVTVSS

SEQ ID NO: 67 - protein, 108 aa, Artificial Sequence
  Synthetic Polypeptide
QDIQMTQSPSSLSASVGDRVTITCRASQSIAIFLNWYQQTPGKPPKLLIYGASTLQSGVPSRFSGSGSGADFTLTISNLQLEDFTTYYCQQSYSTLYTFGQGTKLEIK

SEQ ID NO: 68 - protein, 117 aa, Artificial Sequence
  Synthetic Polypeptide
EVQLLESGGGLVQPGGSLRLSCAASGFTFSRYSMSWVRQAPGKGLEWVSVISSSGGMTYYADSVKGRFTISRDNSKNTLYLQMNSLRAEDTAMYYCARDYYGNMDVWGKGTTVTVSS

SEQ ID NO: 69 - protein, 108 aa, Artificial Sequence
  Synthetic Polypeptide
QDIQMTQSPSSLSTSVGDRVTITCRTSQDISGALAWYQQKPGKAPRLLIFGASSLESGVPSRFSGSGSGTDFTLTISSLQPEDFATYYCQQFNKYPLTFGGGTKVEIK

SEQ ID NO: 70 - protein, 116 aa, Artificial Sequence
  Synthetic Polypeptide
EVQLLESGGGLVQPGGSLRLSCAASGFTFSWYTMGWVRQAPGKGLEWVSYIYPSGGYTMYADSVKGRFTISRDNSKNTLYLQMNSLRAEDTAVYYCANPYSSGGYWGQGTLVTVSS

SEQ ID NO: 71 - protein, 113 aa, Artificial Sequence
  Synthetic Polypeptide
QDIQMTQSPLSLPVTPGEPASISCRSSQSLLDSNGYNYLDWFLQKPGQSPQLLIYLGFNRASGVPDRFSGSGSGTDFTLKISRVEAEDVGVYYCMQALQTPYTFGQGTKLEIT

SEQ ID NO: 72 - protein, 120 aa, Artificial Sequence
  Synthetic Polypeptide
EVQLLESGGGLVQPGGSLRLSCAASGFTFSAYLMTWVRQAPGKGLEWVSGISPSGGITKYADSVKGRFTISRDNSKNTLYLQMNSLRAEDTAVYYCARDIPNWIYGMDVWGQGTTVTVSS

SEQ ID NO: 73 - protein, 105 aa, Artificial Sequence
  Synthetic Polypeptide
QSALTQPPSVSVSPGQTASITCSGDKLGNKYASWYQQKPGQSPVLVIYQDRRRPSGIPERFSGSNSGNTATLTISGTQAMDEADYYCQAWDSGVVFGGGTKLTVL

SEQ ID NO: 74 - protein, 124 aa, Artificial Sequence
  Synthetic Polypeptide
EVQLLESGGGLVQPGGSLRLSCAASGFTFSNYLMLWVRQAPGKGLEWVSGISPSGGGTAYADSVKGRFTISRDNSKNTLYLQMNSLRAEDMAVYYCAKVAYSGSYYYYYYMDVWGKGTTVTVSS

SEQ ID NO: 75 - protein, 109 aa, Artificial Sequence
  Synthetic Polypeptide
QDIQMTQSPSSLSASVGDRVTITCRASQSISSYLNWYQQKPGKAPKLLIYAASSLQSGVPSRFSGSGSGTDFTLTISSLQPEDFATYYCQQSYSTHSITFGQGTRLEIK

SEQ ID NO: 76 - protein, 137 aa, Artificial Sequence
  Synthetic Polypeptide
EVQLLESGGGLVQPGGSLRLSCAASGFTFSQYIMGWVRQAPGKGLEWVSSIGSSGVTVYADSVKGRFTISRDNSKNTLYLQMNSLRAEDTAVYYCARGGGVTVLHAFDIWGQGTMVTVSSASTKGPSVFPLAPSSKS

SEQ ID NO: 77 - protein, 118 aa, Artificial Sequence
  Synthetic Polypeptide
QSALTQPASVSGSPGQSITISCTGTSSDVGGYNYVSWYQQHPGKVPKLIIYEGNKRPSGVPDRFSGSKAGNTASLTVSGLQAEDEADYYCTAYGGHSRFYVFGTGTKVTVLGQPKANP

SEQ ID NO: 78 - protein, 304 aa, Homo sapiens
MIYTMKKVHALWASVCLLLNLAPAPLNADSEEDEEHTIITDTELPPLKLMHSFCAFKADDGPCKAIMKRFFFNIFTRQCEEFIYGGCEGNQNRFESLEECKKMCTRDNANRIIKTTLQQEKPDFCFLEEDPGICRGYITRYFYNNQTKQCERFKYGGCLGNMNNFETLEECKNICEDGPNGFQVDNYGTQLNAVNNSLTPQSTKVPSLFEFHGPSWCLTPADRGLCRANENRFYYNSVIGKCRPFKYSGCGGNENNFTSKQECLRACKKGFIQRISKGGLIKTKRKRKKQRVKIAYEEIFVKNM

SEQ ID NO: 79 - protein, 58 aa, Homo sapiens [sequence omitted]

SEQ ID NO: 80 - protein, 60 aa, Artificial Sequence
  Synthetic Polypeptide
EAMHSFCAFKADDGPCRAAHPRWFFNIFTRQCEEFIYGGCEGNQNRFESLEECKKMCTRD

SEQ ID NO: 81 - protein, 122 aa, Artificial Sequence
  Synthetic Polypeptide
EVQLLESGGGLVQPGGSLRLSCAASGFTFSHYIMMWVRQAPGKGLEWVSGIYSSGGITVYADSVKGRFTISRDNSKNTLYLQMNSLRAEDTAVYYCAYRRIGVPRRDEFDIWGQGTMVTVSS

SEQ ID NO: 82 - protein, 105 aa, Artificial Sequence
  Synthetic Polypeptide
DIQMTQSPSTLSASVGDRVTITCRASQSISSWLAWYQQKPGKAPKLLIYKASTLESGVPSRFSGSGSGTEFTLTISSLQPDDFATYYCQQYNTYWTFGQGTKVEI

SEQ ID NO: 83 - protein, 20 aa, Artificial Sequence
  Synthetic Polypeptide
HKHGHGHGKHKNKGKKNGKH